European Patent Specification EP 3 977 121 B1, published March 19, 2025. Title: A CHEMOENZYMATIC METHOD FOR THE DETECTION OF CELL-CELL PROXIMITY INTERACTION AND ISOLATION OF TUMOR-SPECIFIC ANTIGEN REACTIVE T CELLS FOR IMMUNE THERAPY. Applicant: The Scripps Research Institute Wu, Peng Liu, Zilei Li, Jie Teijaro, John. The sequence listing filed with the application follows.

SEQUENCE LISTING (75 sequences)

SEQ ID NO: 1 - protein, 416 aa, Artificial Sequence
  Made in Lab - FUT6 lentivirus construct
MAKGFYISKSLGILGILLGVAAVCTIIALSVVYSQEKNKNANSSPVASTTPSASATTNPASATTLGGYPYDVPDYAEFASTSLYKKAGSENLYFQGDPTVYPNGSRFPDSTGTPAHSIPLILLWTWPFNKPIALPRCSEMVPGTADCNITADRKVYPQADAVIVHHREVMYNPSAQLPRSPRRQGQRWIWFSMESPSHCWQLKAMDGYFNLTMSYRSDSDIFTPYGWLEPWSGQPAHPPLNLSAKTELVAWAVSNWGPNSARVRYYQSLQAHLKVDVYGRSHKPLPQGTMMETLSRYKFYLAFENSLHPDYITEKLWRNALEAWAVPVVLGPSRSNYERFLPPDAFIHVDDFQSPKDLARYLQELDKDHARYLSYFRWRETLRPRSFSWALAFCKACWKLQEESRYQTRGIAAWFT

SEQ ID NO: 2 - DNA, 1251 bp, Artificial Sequence
  Made in Lab - FUT6 lentivirus construct
atggccaagggcttctatatttccaagtccctgggcatcctggggatcctcctgggcgtggcagccgtgtgcacaatcatcgcactgtcagtggtgtactcccaggagaagaacaagaacgccaacagctcccccgtggcctccaccaccccgtccgcctcagccaccaccaaccccgcctcggccaccaccttgggcggctacccatacgatgttccagattacgctgagttcgccagcaccagcctgtacaagaaggccggcagcgagaacctgtacttccagggcgatcccactgtgtaccctaatgggtcccgcttcccagacagcacagggacccccgcccactccatccccctgatcctgctgtggacgtggccttttaacaaacccatagctctgccccgctgctcagagatggtgcctggcacggctgactgcaacatcactgccgaccgcaaggtgtatccacaggcagacgcggtcatcgtgcaccaccgagaggtcatgtacaaccccagtgcccagctcccacgctccccgaggcggcaggggcagcgatggatctggttcagcatggagtccccaagccactgctggcagctgaaagccatggacggatacttcaatctcaccatgtcctaccgcagcgactccgacatcttcacgccctacggctggctggagccgtggtccggccagcctgcccacccaccgctcaacctctcggccaagaccgagctggtggcctgggcagtgtccaactgggggccaaactccgccagggtgcgctactaccagagcctgcaggcccatctcaaggtggacgtgtacggacgctcccacaagcccctgccccagggaaccatgatggagacgctgtcccggtacaagttctatctggccttcgagaactccttgcaccccgactacatcaccgagaagctgtggaggaacgccctggaggcctgggccgtgcccgtggtgctgggccccagcagaagcaactacgagaggttcctgccacccgacgccttcatccacgtggacgacttccagagccccaaggacctggcccggtacctgcaggagctggacaaggaccacgcccgctacctgagctactttcgctggcgggagacgctgcggcctcgctccttcagctgggcactcgctttctgcaaggcctgctggaaactgcaggaggaatccaggtaccagacacgcggcatagcggcttggttcacctga

SEQ ID NO: 3 - DNA, 8622 bp, Artificial Sequence
  Made in Lab - lentivirus expression vector
caggtggcacttttcggggaaatgtgcgcggaacccctatttgtttatttttctaaatacattcaaatatgtatccgctcatgagacaataaccctgataaatgcttcaataatattgaaaaaggaagagtatgagtattcaacatttccgtgtcgcccttattcccttttttgcggcattttgccttcctgtttttgctcacccagaaacgctggtgaaagtaaaagatgctgaagatcagttgggtgcacgagtgggttacatcgaactggatctcaacagcggtaagatccttgagagttttcgccccgaagaacgttttccaatgatgagcacttttaaagttctgctatgtggcgcggtattatcccgtattgacgccgggcaagagcaactcggtcgccgcatacactattctcagaatgacttggttgagtactcaccagtcacagaaaagcatcttacggatggcatgacagtaagagaattatgcagtgctgccataaccatgagtgataacactgcggccaacttacttctgacaacgatcggaggaccgaaggagctaaccgcttttttgcacaacatgggggatcatgtaactcgccttgatcgttgggaaccggagctgaatgaagccataccaaacgacgagcgtgacaccacgatgcctgtagcaatggcaacaacgttgcgcaaactattaactggcgaactacttactctagcttcccggcaacaattaatagactggatggaggcggataaagttgcaggaccacttctgcgctcggcccttccggctggctggtttattgctgataaatctggagccggtgagcgtgggtctcgcggtatcattgcagcactggggccagatggtaagccctcccgtatcgtagttatctacacgacggggagtcaggcaactatggatgaacgaaatagacagatcgctgagataggtgcctcactgattaagcattggtaactgtcagaccaagtttactcatatatactttagattgatttaaaacttcatttttaatttaaaaggatctaggtgaagatcctttttgataatctcatgaccaaaatcccttaacgtgagttttcgttccactgagcgtcagaccccgtagaaaagatcaaaggatcttcttgagatcctttttttctgcgcgtaatctgctgcttgcaaacaaaaaaaccaccgctaccagcggtggtttgtttgccggatcaagagctaccaactctttttccgaaggtaactggcttcagcagagcgcagataccaaatactgtccttctagtgtagccgtagttaggccaccacttcaagaactctgtagcaccgcctacatacctcgctctgctaatcctgttaccagtggctgctgccagtggcgataagtcgtgtcttaccgggttggactcaagacgatagttaccggataaggcgcagcggtcgggctgaacggggggttcgtgcacacagcccagcttggagcgaacgacctacaccgaactgagatacctacagcgtgagctatgagaaagcgccacgcttcccgaagggagaaaggcggacaggtatccggtaagcggcagggtcggaacaggagagcgcacgagggagcttccagggggaaacgcctggtatctttatagtcctgtcgggtttcgccacctctgacttgagcgtcgatttttgtgatgctcgtcaggggggcggagcctatggaaaaacgccagcaacgcggcctttttacggttcctggccttttgctggccttttgctcacatgttctttcctgcgttatcccctgattctgtggataaccgtattaccgcctttgagtgagctgataccgctcgccgcagccgaacgaccgagcgcagcgagtcagtgagcgaggaagcggaagagcgcccaatacgcaaaccgcctctccccgcgcgttggccgattcattaatgcagctggcacgacaggtttcccgactggaaagcgggcagtgagcgcaacgcaattaatgtgagttagctcactcattaggcaccccaggctttacactttatgcttccggctcgtatgttgtgtggaattgtgagcggataacaatttcacacaggaaacagctatgaccatgattacgccaagcgcgcaattaaccctcactaaagggaacaaaagctggagctgcaagcttaatgtagtcttatgcaatactcttgtagtcttgcaacatggtaacgatgagttagcaacatgccttacaaggagagaaaaagcaccgtgcatgccgattggtggaagtaaggtggtacgatcgtgccttattaggaaggcaacagacgggtctgacatggattggacgaaccactgaattgccgcattgcagagatattgtatttaagtgcctagctcgatacaataaacgggtctctctggttagaccagatctgagcctgggagctctctggctaactagggaacccactgcttaagcctcaataaagcttgccttgagtgcttcaagtagtgtgtgcccgtctgttgtgtgactctggtaactagagatccctcagacccttttagtcagtgtggaaaatctctagcagtggcgcccgaacagggacctgaaagcgaaagggaaaccagagctctctcgacgcaggactcggcttgctgaagcgcgcacggcaagaggcgaggggcggcgactggtgagtacgccaaaaattttgactagcggaggctagaaggagagagatgggtgcgagagcgtcagtattaagcgggggagaattagatcgcgatgggaaaaaattcggttaaggccagggggaaagaaaaaatataaattaaaacatatagtatgggcaagcagggagctagaacgattcgcagttaatcctggcctgttagaaacatcagaaggctgtagacaaatactgggacagctacaaccatcccttcagacaggatcagaagaacttagatcattatataatacagtagcaaccctctattgtgtgcatcaaaggatagagataaaagacaccaaggaagctttagacaagatagaggaagagcaaaacaaaagtaagaccaccgcacagcaagcggccgctgatcttcagacctggaggaggagatatgagggacaattggagaagtgaattatataaatataaagtagtaaaaattgaaccattaggagtagcacccaccaaggcaaagagaagagtggtgcagagagaaaaaagagcagtgggaataggagctttgttccttgggttcttgggagcagcaggaagcactatgggcgcagcctcaatgacgctgacggtacaggccagacaattattgtctggtatagtgcagcagcagaacaatttgctgagggctattgaggcgcaacagcatctgttgcaactcacagtctggggcatcaagcagctccaggcaagaatcctggctgtggaaagatacctaaaggatcaacagctcctggggatttggggttgctctggaaaactcatttgcaccactgctgtgccttggaatgctagttggagtaataaatctctggaacagattggaatcacacgacctggatggagtgggacagagaaattaacaattacacaagcttaatacactccttaattgaagaatcgcaaaaccagcaagaaaagaatgaacaagaattattggaattagataaatgggcaagtttgtggaattggtttaacataacaaattggctgtggtatataaaattattcataatgatagtaggaggcttggtaggtttaagaatagtttttgctgtactttctatagtgaatagagttaggcagggatattcaccattatcgtttcagacccacctcccaaccccgaggggacccgacaggcccgaaggaatagaagaagaaggtggagagagagacagagacagatccattcgattagtgaacggatctcgacggttaacttttaaaagaaaaggggggattggggggtacagtgcaggggaaagaatagtagacataatagcaacagacatacaaactaaagaattacaaaaacaaattacaaaaattcaaaattttatcgagctttgcaaagatggataaagttttaaacagagaggaatctttgcagctaatggaccttctaggtcttgaaaggagtgcctcgtgaggctccggtgcccgtcagtgggcagagcgcacatcgcccacagtccccgagaagttggggggaggggtcggcaattgaaccggtgcctagagaaggtggcgcggggtaaactgggaaagtgatgtcgtgtactggctccgcctttttcccgagggtgggggagaaccgtatataagtgcagtagtcgccgtgaacgttctttttcgcaacgggtttgccgccagaacacaggtaagtgccgtgtgtggttcccgcgggcctggcctctttacgggttatggcccttgcgtgccttgaattacttccacctggctgcagtacgtgattcttgatcccgagcttcgggttggaagtgggtgggagagttcgaggccttgcgcttaaggagccccttcgcctcgtgcttgagttgaggcctggcctgggcgctggggccgccgcgtgcgaatctggtggcaccttcgcgcctgtctcgctgctttcgataagtctctagccatttaaaatttttgatgacctgctgcgacgctttttttctggcaagatagtcttgtaaatgcgggccaagatctgcacactggtatttcggtttttggggccgcgggcggcgacggggcccgtgcgtcccagcgcacatgttcggcgaggcggggcctgcgagcgcggccaccgagaatcggacgggggtagtctcaagctggccggcctgctctggtgcctggcctcgcgccgccgtgtatcgccccgccctgggcggcaaggctggcccggtcggcaccagttgcgtgagcggaaagatggccgcttcccggccctgctgcagggagctcaaaatggaggacgcggcgctcgggagagcgggcgggtgagtcacccacacaaaggaaaagggcctttccgtcctcagccgtcgcttcatgtgactccacggagtaccgggcgccgtccaggcacctcgattagttctcgagcttttggagtacgtcgtctttaggttggggggaggggttttatgcgatggagtttccccacactgagtgggtggagactgaagttaggccagcttggcacttgatgtaattctccttggaatttgccctttttgagtttggatcttggttcattctcaagcctcagacagtggttcaaagtttttttcttccatttcaggtgtcgtgaggaattcggtaccgcggccgcccggggatccatggccaagggcttctatatttccaagtccctgggcatcctggggatcctcctgggcgtggcagccgtgtgcacaatcatcgcactgtcagtggtgtactcccaggagaagaacaagaacgccaacagctcccccgtggcctccaccaccccgtccgcctcagccaccaccaaccccgcctcggccaccaccttgggcggctacccatacgatgttccagattacgctgagttcgccagcaccagcctgtacaagaaggccggcagcgagaacctgtacttccagggcgatcccactgtgtaccctaatgggtcccgcttcccagacagcacagggacccccgcccactccatccccctgatcctgctgtggacgtggccttttaacaaacccatagctctgccccgctgctcagagatggtgcctggcacggctgactgcaacatcactgccgaccgcaaggtgtatccacaggcagacgcggtcatcgtgcaccaccgagaggtcatgtacaaccccagtgcccagctcccacgctccccgaggcggcaggggcagcgatggatctggttcagcatggagtccccaagccactgctggcagctgaaagccatggacggatacttcaatctcaccatgtcctaccgcagcgactccgacatcttcacgccctacggctggctggagccgtggtccggccagcctgcccacccaccgctcaacctctcggccaagaccgagctggtggcctgggcagtgtccaactgggggccaaactccgccagggtgcgctactaccagagcctgcaggcccatctcaaggtggacgtgtacggacgctcccacaagcccctgccccagggaaccatgatggagacgctgtcccggtacaagttctatctggccttcgagaactccttgcaccccgactacatcaccgagaagctgtggaggaacgccctggaggcctgggccgtgcccgtggtgctgggccccagcagaagcaactacgagaggttcctgccacccgacgccttcatccacgtggacgacttccagagccccaaggacctggcccggtacctgcaggagctggacaaggaccacgcccgctacctgagctactttcgctggcgggagacgctgcggcctcgctccttcagctgggcactcgctttctgcaaggcctgctggaaactgcaggaggaatccaggtaccagacacgcggcatagcggcttggttcacctgagtcgacaatcaacctctggattacaaaatttgtgaaagattgactggtattcttaactatgttgctccttttacgctatgtggatacgctgctttaatgcctttgtatcatgctattgcttcccgtatggctttcattttctcctccttgtataaatcctggttgctgtctctttatgaggagttgtggcccgttgtcaggcaacgtggcgtggtgtgcactgtgtttgctgacgcaacccccactggttggggcattgccaccacctgtcagctcctttccgggactttcgctttccccctccctattgccacggcggaactcatcgccgcctgccttgcccgctgctggacaggggctcggctgttgggcactgacaattccgtggtgttgtcggggaagctgacgtcctttccatggctgctcgcctgtgttgccacctggattctgcgcgggacgtccttctgctacgtcccttcggccctcaatccagcggaccttccttcccgcggcctgctgccggctctgcggcctcttccgcgtcttcgccttcgccctcagacgagtcggatctccctttgggccgcctccccgcctggaattcgagctcggtacctttaagaccaatgacttacaaggcagctgtagatcttagccactttttaaaagaaaaggggggactggaagggctaattcactcccaacgaagacaagatctgctttttgcttgtactgggtctctctggttagaccagatctgagcctgggagctctctggctaactagggaacccactgcttaagcctcaataaagcttgccttgagtgcttcaagtagtgtgtgcccgtctgttgtgtgactctggtaactagagatccctcagacccttttagtcagtgtggaaaatctctagcagtagtagttcatgtcatcttattattcagtatttataacttgcaaagaaatgaatatcagagagtgagaggaacttgtttattgcagcttataatggttacaaataaagcaatagcatcacaaatttcacaaataaagcatttttttcactgcattctagttgtggtttgtccaaactcatcaatgtatcttatcatgtctggctctagctatcccgcccctaactccgcccagttccgcccattctccgccccatggctgactaattttttttatttatgcagaggccgaggccgcctcggcctctgagctattccagaagtagtgaggaggcttttttggaggcctaggcttttgcgtcgagacgtacccaattcgccctatagtgagtcgtattacgcgcgctcactggccgtcgttttacaacgtcgtgactgggaaaaccctggcgttacccaacttaatcgccttgcagcacatccccctttcgccagctggcgtaatagcgaagaggcccgcaccgatcgcccttcccaacagttgcgcagcctgaatggcgaatggcgcgacgcgccctgtagcggcgcattaagcgcggcgggtgtggtggttacgcgcagcgtgaccgctacacttgccagcgccctagcgcccgctcctttcgctttcttcccttcctttctcgccacgttcgccggctttccccgtcaagctctaaatcgggggctccctttagggttccgatttagtgctttacggcacctcgaccccaaaaaacttgattagggtgatggttcacgtagtgggccatcgccctgatagacggtttttcgccctttgacgttggagtccacgttctttaatagtggactcttgttccaaactggaacaacactcaaccctatctcggtctattcttttgatttataagggattttgccgatttcggcctattggttaaaaaatgagctgatttaacaaaaatttaacgcgaattttaacaaaatattaacgtttacaatttcc

SEQ ID NO: 4 - protein, 5 aa, Unknown
  Sortase recognition sequence motif
  misc_feature (3)..(3): Xaa can be any naturally occurring amino acid
  MOD_RES (5)..(5): Xaa is any amino acid residue
LPXTX

SEQ ID NO: 5 - protein, 5 aa, Unknown
  Sortase recognition sequence
LPETG

SEQ ID NO: 6 - protein, 5 aa, Unknown
  Modified sortase recognition sequence motif
  MOD_RES (3)..(3): Xaa is any amino acid residue
LAXTG

SEQ ID NO: 7 - protein, 5 aa, Unknown
  Modified sortase recognition sequence motif
  MOD_RES (3)..(3): Xaa is any amino acid residue
LAXSG

SEQ ID NO: 8 - protein, 5 aa, Unknown
  Sortase recognition sequence
LPKTG

SEQ ID NO: 9 - protein, 5 aa, Unknown
  Sortase recognition sequence
LPATG

SEQ ID NO: 10 - protein, 5 aa, Unknown
  Sortase recognition sequence
LPNTG

SEQ ID NO: 11 - protein, 5 aa, Unknown
  Sortase recognition sequence
  MOD_RES (3)..(3): Xaa is any amino acid residue
LPXAG

SEQ ID NO: 12 - protein, 5 aa, Unknown
  Sortase recognition sequence
LPNAG

SEQ ID NO: 13 - protein, 5 aa, Unknown
  Sortase recognition sequence
  MOD_RES (3)..(3): Xaa is any amino acid residue
LPXTA

SEQ ID NO: 14 - protein, 5 aa, Unknown
  Sortase recognition sequence
LPNTA

SEQ ID NO: 15 - protein, 5 aa, Unknown
  Sortase recognition sequence
  MOD_RES (3)..(3): Xaa is any amino acid residue
LGXTG

SEQ ID NO: 16 - protein, 5 aa, Unknown
  Sortase recognition sequence
LGATG

SEQ ID NO: 17 - protein, 5 aa, Unknown
  Sortase recognition sequence
  MOD_RES (3)..(3): Xaa is any amino acid residue
IPXTG

SEQ ID NO: 18 - protein, 5 aa, Unknown
  Sortase recognition sequence
IPNTG

SEQ ID NO: 19 - protein, 5 aa, Unknown
  Sortase recognition sequence
IPETG

SEQ ID NO: 20 - protein, 5 aa, Unknown
  Sortase recognition sequence
LAETG

SEQ ID NO: 21 - protein, 5 aa, Unknown
  Sortase recognition sequence motif
  MOD_RES (3)..(3): Xaa is Q or K
  MOD_RES (4)..(4): Xaa is T or S
  MOD_RES (5)..(5): Xaa is N, G or S
NPXXX

SEQ ID NO: 22 - protein, 5 aa, Unknown
  Sortase recognition sequence
  MOD_RES (3)..(3): Xaa is any amino acid residue
NPQTN

SEQ ID NO: 23 - protein, 5 aa, Unknown
  Sortase recognition sequence
NPKTG

SEQ ID NO: 24 - protein, 5 aa, Unknown
  Sortase recognition sequence
  MOD_RES (3)..(3): Xaa is any amino acid residue
NSKTA

SEQ ID NO: 25 - protein, 5 aa, Unknown
  Sortase recognition sequence
NPQTG

SEQ ID NO: 26 - protein, 5 aa, Unknown
  Sortase recognition sequence
NAKTN

SEQ ID NO: 27 - protein, 5 aa, Unknown
  Sortase recognition sequence
NPQSS

SEQ ID NO: 28 - protein, 5 aa, Unknown
  Sortase recognition sequence motif
  MOD_RES (4)..(4): Xaa is any amino acid residue
LPTXG

SEQ ID NO: 29 - protein, 10 aa, Artificial Sequence
  Made in Lab - complementarity determining region sequence
ASGTDYAEQF

SEQ ID NO: 30 - protein, 13 aa, Artificial Sequence
  Made in Lab - complementarity determining region sequence
ASSPQLGGRREQY

SEQ ID NO: 31 - protein, 12 aa, Artificial Sequence
  Made in Lab - complementarity determining region sequence
ASSIGTANTEVF

SEQ ID NO: 32 - protein, 9 aa, Artificial Sequence
  Made in Lab - complementarity determining region sequence
AWSGNTEVF

SEQ ID NO: 33 - protein, 12 aa, Artificial Sequence
  Made in Lab - complementarity determining region sequence
ASRSGGSAETLY

SEQ ID NO: 34 - protein, 12 aa, Artificial Sequence
  Made in Lab - complementarity determining region sequence
ASSFVSSAETLY

SEQ ID NO: 35 - protein, 13 aa, Artificial Sequence
  Made in Lab - complementarity determining region sequence
ASSSDRGSAETLY

SEQ ID NO: 36 - protein, 12 aa, Artificial Sequence
  Made in Lab - complementarity determining region sequence
ASSDRGGQDTQY

SEQ ID NO: 37 - protein, 11 aa, Artificial Sequence
  Made in Lab - complementarity determining region sequence
ASSSGTDTEVF

SEQ ID NO: 38 - protein, 11 aa, Artificial Sequence
  Made in Lab - complementarity determining region sequence
AWRDWGGAEQF

SEQ ID NO: 39 - protein, 10 aa, Artificial Sequence
  Made in Lab - complementarity determining region sequence
ASSGLGETLY

SEQ ID NO: 40 - protein, 12 aa, Artificial Sequence
  Made in Lab - complementarity determining region sequence
ASSLDNSGNTLY

SEQ ID NO: 41 - protein, 12 aa, Artificial Sequence
  Made in Lab - complementarity determining region sequence
ASSLDRVQDTQY

SEQ ID NO: 42 - protein, 6 aa, Artificial Sequence
  Made in Lab - complementarity determining region sequence
AWTEVF

SEQ ID NO: 43 - protein, 12 aa, Artificial Sequence
  Made in Lab - complementarity determining region sequence
ASSFGQNYAEQF

SEQ ID NO: 44 - protein, 12 aa, Artificial Sequence
  Made in Lab - complementarity determining region sequence
ASSDGTSAETLY

SEQ ID NO: 45 - protein, 11 aa, Artificial Sequence
  Made in Lab - complementarity determining region sequence
ASRPGSAETLY

SEQ ID NO: 46 - protein, 10 aa, Artificial Sequence
  Made in Lab - complementarity determining region sequence
ASSPQLYEQY

SEQ ID NO: 47 - protein, 14 aa, Artificial Sequence
  Made in Lab - complementarity determining region sequence
ASSDGLGVNQDTQY

SEQ ID NO: 48 - protein, 12 aa, Artificial Sequence
  Made in Lab - complementarity determining region sequence
ASSDGGGGTEVF

SEQ ID NO: 49 - protein, 13 aa, Artificial Sequence
  Made in Lab - complementarity determining region sequence
AWSLRLGGTYEQY

SEQ ID NO: 50 - protein, 12 aa, Artificial Sequence
  Made in Lab - complementarity determining region sequence
ASSLTISNERLF

SEQ ID NO: 51 - protein, 12 aa, Artificial Sequence
  Made in Lab - complementarity determining region sequence
ASSFWGRQDTQY

SEQ ID NO: 52 - protein, 12 aa, Artificial Sequence
  Made in Lab - complementarity determining region sequence
ASSFWGRGNTLY

SEQ ID NO: 53 - protein, 13 aa, Artificial Sequence
  Made in Lab - complementarity determining region sequence
ASGGPGQGFAEQF

SEQ ID NO: 54 - protein, 11 aa, Artificial Sequence
  Made in Lab - complementarity determining region sequence
ASSPTGAIMNS

SEQ ID NO: 55 - protein, 14 aa, Artificial Sequence
  Made in Lab - complementarity determining region sequence
ASSLYRDRGYAEQF

SEQ ID NO: 56 - protein, 13 aa, Artificial Sequence
  Made in Lab - complementarity determining region sequence
AWSLPLGQSYEQY

SEQ ID NO: 57 - protein, 10 aa, Artificial Sequence
  Made in Lab - complementarity determining region sequence
ASSFRGYEQY

SEQ ID NO: 58 - protein, 10 aa, Artificial Sequence
  Made in Lab - complementarity determining region sequence
ASSDDTYEQY

SEQ ID NO: 59 - protein, 11 aa, Artificial Sequence
  Made in Lab - complementarity determining region sequence
ASSDGDRYEQY

SEQ ID NO: 60 - protein, 11 aa, Artificial Sequence
  Made in Lab - complementarity determining region sequence
ASSDNYNSPLY

SEQ ID NO: 61 - protein, 13 aa, Artificial Sequence
  Made in Lab - complementarity determining region sequence
ASRDWGGRAETLY

SEQ ID NO: 62 - protein, 12 aa, Artificial Sequence
  Made in Lab - complementarity determining region sequence
ASSLELGGREQY

SEQ ID NO: 63 - protein, 13 aa, Artificial Sequence
  Made in Lab - complementarity determining region sequence
ASSDPGAANTEVF

SEQ ID NO: 64 - protein, 12 aa, Artificial Sequence
  Made in Lab - complementarity determining region sequence
ASSLDGADSDYT

SEQ ID NO: 65 - protein, 10 aa, Artificial Sequence
  Made in Lab - complementarity determining region sequence
ASSMNNERLF

SEQ ID NO: 66 - protein, 13 aa, Artificial Sequence
  Made in Lab - complementarity determining region sequence
ASSQVGGASETLY

SEQ ID NO: 67 - protein, 14 aa, Artificial Sequence
  Made in Lab - complementarity determining region sequence
ASGDATDYSGNTLY

SEQ ID NO: 68 - protein, 12 aa, Artificial Sequence
  Made in Lab - complementarity determining region sequence
ASGEGPANTEVF

SEQ ID NO: 69 - protein, 8 aa, Gallus gallus
SIINFEKL

SEQ ID NO: 70 - protein, 8 aa, Artificial Sequence
  Made in Lab - Altered ovalbumin peptide
SAINFEKL

SEQ ID NO: 71 - protein, 8 aa, Artificial Sequence
  Made in Lab - Altered ovalbumin peptide
SIITFEKL

SEQ ID NO: 72 - protein, 20 aa, Lymphocytic choriomeningitis virus
GLNGPDIYKGVYQFKSVEFD

SEQ ID NO: 73 - protein, 9 aa, Homo sapiens
KVPRNQDWL

SEQ ID NO: 74 - protein, 9 aa, Macaca mulatta polyomavirus
SAINNYAQK

SEQ ID NO: 75 - protein, 9 aa, Lymphocytic choreomeningitis virus
KAVYNFATM